European Patent Application EP 4 170 037 A1, published April 26, 2023. Title: Salmonella strain for treating cancer and use thereof. Applicant: Industry Foundation of Channam National University. The sequence listing filed with the application follows.

SEQUENCE LISTING (15 sequences)

SEQ ID NO: 1 - DNA, 35012 bp, Unknown
  Salmonella pathogenicity island-1
taattatatcatgatgagttcagccaacggtgatatggccttataaggcttgcagtctttcatgggcagcaagtaacgtctgatatatgcttaaattcttacttccgggttcaagcaaaacttttttaaattcggtcatgagttgctcttcatcttctttcgaacgcatgtattgtggatgttcctggaagaaggtgagcgcctgttctttggtttgtttatatttttcgcaaaaaatgcttgagctgattgcgctattttttgatgcggaattatcagcgttatggtttgataatgatttattcttcgcaaggtctgacggcacatacggaagagactgacactcatcaatactatttgcgttggccagttgctctttctgagcgccaggttgctgtaccggtttgctcacggaggaagggaggggcacctgagcacagccgatcagtaaaaagacaggaagacagctataaaattttttcatattaactccaactacagaagaatgaggcgccatgtttttacacaaccgtcagaacgttatctgacaatagttataagggggcgaatgcgtttcaggaatgctagcaaaaaaaactcctgatataaataattaattctccatccagatgacaatatctgaatttttgctgctgcagaacaataagccagaatttatacactatgagctaattttctattttaaatcagcaaacactatgcaagttggccaatttaattagcgggcggcatcagtttcataatgattgcatcaggattttgccacccgctcccggtattgtttacatattaaaatgatttttaactggtgctgacaactatgctaaatacgcaggaagtacttaaagaaggagagaagcggaaaatccgcagcccggaagcatggtttatacagacgtgttccgcgcaaaagctgcatatgtcattttctgaaagccgacacaatgaaaattgcctgattcaggaaggcgcgctgcttttttgcgagcaggccgttgtcgcaccagtatcaggagacctggtttttcgaccgttaaaaattgaagtactcagcaaattactggcatttatcgatggcgcaggattagtggacacgacatatgctgaatccgataaatgggttttgctgagtcctgagtttcgcgctatttggcaagatcgtaaacgctgcgagtactggtttttgcagcaaattattacgccttctccggccttcaataaggtactggcgctgttacgaaaaagcgagagttactggttggttggctatttactcgctcagtcaaccagcggcaacacgatgagaatgctgggagaagactatggcgtttcttatacccattttcgtcgtttgtgcagcagagcgttgggcggaaaagcgaagagtgaattacgaaactggcgtatggcgcaatcgctgctgaatagtgtagaaggccacgagaacatcacccaattagccgttaatcatggttactcatcgccttcacatttttctagtgagatcaaagagctgatcggcgtttcgccgcggaaattatcaaatattattcaattggcagacaaatgaagacacatattcttttggccagagtgctggcatgtgccgcgcttgttctggttacacctggttattctagtgaaaaaatacctgtaacgggaagtgggtttgttgcgaaagacgatagcctgcggacatttttcgatgccatggcgctacagctaaaggagcctgtcattgttagcaaaatggcggcacgaaaaaaaattacgggcaactttgagtttcacgatcctaacgcattactggagaagctttccctacaactggggctgatttggtatttcgatgggcaggctatctatatttatgacgccagtgaaatgcgcaatgccgtggtttctttacgcaacgtctcactcaatgagttcaacaattttctaaaacgctcaggtttatataacaaaaattacccgctacgtggcgataaccgtaaaggaacattctatgtttcagggccacccgtctatgttgatatggtggtcaacgccgccaccatgatggacaagcaaaacgatggtattgagctgggacgccagaaaataggggtgatgcgtctgaacaataccttcgtgggcgatcgtacctataatctgcgcgatcagaaaatggttattcccggtattgctacggccattgaaaggttattgcagggagaagagcaacccttaggtaatattgtcagtagcgaacccccggcgatgccagcgttttcagcgaatggagaaaaaggtaaagcagcaaattatgccggtggcatgagtctgcaggaagctttaaagcaaaatgccgcggcgggcaatattaaaatcgtggcctatccggataccaacagtttgttagtaaagggaacggctgagcaggtgcattttatcgaaatgctggttaaagcgctggatgtcgccaaacgtcacgtagaattatccctgtggattgtcgatcttaataaaagcgatctggagcgtttgggcacttcatggagcggcagcataactattggggacaaacttggcgtgtcattaaaccagtcttcaataagtaccctcgatggcagtcgattcatcgccgcggtcaatgcgttagaagagaagaaacaggcgacggtggtttcgcgcccggtattactgactcaggaaaatgttcccgctatttttgataacaacagaacgttttacaccaagctgattggggaacgtaatgtggcgcttgagcatgtaacatacggaacaatgatccgagtgctgccccgtttttccgcagatggtcagatagaaatgtcgctggacattgaagatggcaacgataagacgccgcaatctgatactaccacctccgtagatgcgttacccgaagtcgggcgaacgttaattagcactattgcgagagtgccgcacggaaaaagtttgctggtcgggggttatacacgggatgcaaataccgatactgtccaaagtattccgtttttaggcaaattaccgcttattggtagcctgttccgttattccagtaagaataaaagtaatgttgttcgtgtgttcatgattgaaccaaaagaaattgtcgacccgttaacgccggatgccagcgaatcggtaaacaatattctgaagcaaagcggtgcctggagtggggacgataagttacagaaatgggttcgtgtttatctggatagaggtcaggaggcaattaaatgattcctggctcaacctccggtatttcattttccagaatattgtcccggcagacatctcatcaggatgcgacccagcatactgatgcgcaacaggcggaaatacaacaggccgcagaggattcgtctccaggggcggaagtacaaaaatttgtccagtcgacggacgaaatgtcagcggcgctggcgcaatttcgtaaccgtcgcgattatgaaaaaaaatccagtaatttatctaacagttttgaacgcgtgctggaggatgaggctttaccgaaggcgaagcaaatcttaaagctaattagcgtacatggcggcgcgttagaagattttttacgtcaggcgcgtagcttatttcctgaccccagtgatttagtccttgtgttacgcgaattgcttcgtcgtaaagacctggaagagatcgtgcggaaaaagctggagtcgttacttaagcacgttgaagagcaaaccgatccgaagaccctcaaggcagggattaattgtgcgttgaaggcccggctttttgggaaaacattatcgttaaaaccaggcttattgcgcgccagctatcggcaatttatccagagtgaatcacatgaagtggagatttactctgactggatagccagttatggctatcaacgtcgactggtggtactggattttattgagggttcgctattaaccgatattgacgcgaatgacgccagctgttcgcgcctggagtttggccagcttttacgacgcctgacgcaacttaaaatgttgcgctccgctgacctactgtttgtgagtacattgttgtcgtattcgtttaccaaagcgtttaatgcggaggagtcgtcgtggttactactgatgctttcgctattgcaacagccacatgaagtggattcgctgttagccgatattataggtttgaatgcgttattgcttagtcataaagaacatgcatcctttttgcagatattttatcaagtatgtaaagccataccctcttcactcttttatgaagaatattggcaggaagaattgttaatggcgttacgtagtatgaccgatattgcctacaagcatgaaatggcagaacagcgtcgtactattgaaaagctgtcttaatttaatattaacaggatacctatagtgctgctttctctacttaacagtgctcgtttacgacctgaattactgattctggtactaatggtgatgatcatttctatgttcgtcattccattacctacctatctggttgatttcctgatcgcactgaatatcgtactggcgatattggtgtttatggggtcgttctacattgacagaatcctcagtttttcaacgtttcctgcggtactgttaattaccacgctctttcgtctggcattatcgatcagtaccagtcgtcttatcttgattgaagccgatgccggtgaaattatcgccacgttcgggcaattcgttattggcgatagcctggcggtgggttttgttgtcttctctattgtcaccgtggtccagtttatcgttattaccaaaggttcagaacgtgtcgcggaagtcgcggcccgattttctctggatggtatgcccggtaaacagatgagtattgatgccgatttgaaggccggtattattgatgcggatgccgcgcgcgaacggcgaagcgtactggaaagggaaagccagctttacggttcctttgacggtgcgatgaagtttatcaaaggtgacgctattgccggcatcattattatctttgtgaactttattggcggtatttcggtggggatgactcgccatggtatggatttgtcctccgccctgtctacttataccatgctgaccattggtgatggtcttgtcgcccagatccccgcattgttgattgcgattagtgccggttttatcgtgacccgcgtaaatggcgatagcgataatatggggcggaatatcatgacgcagctgttgaacaacccatttgtattggttgttacggctattttgaccatttcaatgggaactctgccgggattcccactgccggtttttgttattttatcggtggttttaagcgtactcttctattttaaattccgtgaagcaaaacgtagcgccgccaaacctaaaaccagcaaaggcgagcagccgctcagtattgaggaaaaagaagggtcgtcgttaggactgattggcgatctcgataaagtctctacagagaccgtaccgttgatattacttgtgccgaagagccggcgtgaagatctggaaaaagctcaacttgcggagcgtctacgtagtcagttctttattgattatggcgtgcgcctgccggaagtattgttacgagatggcgagggcctggacgataacagcatcgtattgttgattaatgagatccgtgttgaacaatttacggtctattttgatttgatgcgagtggtaaattattccgatgaagtcgtgtcctttggtattaatccaacaatccatcagcaaggtagcagtcagtatttctgggtaacgcatgaagagggggagaaactccgggagcttggctatgtgttgcggaacgcgcttgatgagctttaccactgtctggcggtgacgctggcgcgcaacgtcaatgaatatttcggtattcaggaaacaaaacatatgctggaccaactggaagcgaaatttcctgatttacttaaagaagtgctcagacatgccacggtacaacgtatatctgaagttttgcagcgtttgttaagcgaacgtgtttccgtgcgtaatatgaagttaattatggaagcgctcgcattgtgggcgccaagagaaaaagatgtcattaaccttgtggagcatattcgtggagcaatggcgcgttatatttgtcataaattcgccaatggcggcgaattacgagcagtaatggtatctgctgaagttgaggatgttattcgcaaagggatccgtcagacctctggcagtaccttcctcagccttgacccggaagcctccgctaatttgatggatctcattacacttaagttggatgatttattgattgcacataaagatcttgtcctccttacgtctgtcgatgtccgtcgatttattaagaaaatgattgaaggtcgttttccggatctggaggttttatctttcggtgagatagcagatagcaagtcagtgaatgttataaaaacaatataagggcttaattaaggaaaagatctatgcaacatttggatatcgctgaattagttcgttccgcactggaagtaagtggttgcgatccttcattaattggaggaatagatagccattcaacaattgttctggatttatttgcattgccaagtatctgtatcagcgtcaaggacgatgatgtatggatctgggcgcaattgggtgctgacagcatggtggtattacaacagcgggcttatgaaatcttaatgaccataatggaaggatgccattttgcccgcggcgggcaattactactgggggagcagaatggggagctaacgcttaaagccttagtgcatccggattttttatctgacggtgaaaagttctctactgccttgaatgggttttacaactatctggaagtttttagtcggtcgctaatgagatgaaaacacctcgtttactgcaatatctggcctacccacaaaaaataaccggcccaattattgaggcggaattgcgcgatgtggccattggcgaactgtgtgaaatacgccgtggctggcaccaaaaacaggttgttgcacgtgcgcaggtggttggcttacagcgggaacgcaccgtgctgagccttatcggcaatgcccaggggctgagccgcgatgtcgtgctttatcccactggacgtgcgttatcggcgtgggtgggatactcggtattaggcgcggtgttggatccgacagggaaaatcgttgagcgttttacccctgaagtggcgccgattagcgaagaacgcgttattgatgtcgcaccgccgtcttacgcttcacgcgttggcgtccgtgaaccgctgattaccggtgtgcgcgcgattgacgggttattgacctgtggcgtaggccagcgaatgggcatttttgcctccgcaggatgcggtaagaccatgctgatgcatatgctgatcgagcaaacggaggcggatgtctttgttatcggtcttatcggtgaacgaggccgtgaggtcactgaattcgtggatatgttgcgcgcttcgcataagaaagaaaaatgcgtgctggtttttgccacttccgatttcccctcggtcgatcgctgcaatgcggcgcaactggcgacaaccgtagcggaatattttcgcgaccagggaaaacgggtcgtgctttttatcgattccatgacccgttatgcgcgtgctttgcgagacgtggcactggcgtcgggagagcgtccggctcgtcgaggttatcccgcctccgtattcgataatttgccccgcttgctggaacgcccaggggcgaccagcgagggaagcattactgccttttatacggtactgctggaaagcgaggaagaggcggacccgatggcggatgaaattcgctctatccttgacggtcacctgtatctgagcagaaagctggccgggcagggacattacccggcaatcgatgtactgaaaagcgtaagccgcgtttttggacaagtcacgacgccgacacatgctgaacaggcatctgccgtgcgtaaattaatgacgcgtttggaagagctccagcttttcattgacttgggagaatatcgtcctggcgaaaatatcgataacgatcgggcgatgcagatgcgggatagcctgaaagcctggttatgccagccggtagcgcagtattcatcctttgatgacacgttgagcggtatgaatgcattcgctgaccagaattaaagtattgcagcggcgctgtacggtatttcattcacagtgtgagtcgatattacttcgctatcaggatgaggaccgcgggctgcaggccgaggaggaggcgatccttgaacaaatagcgggtctgaaattgttattagatacgctgcgtgcagaaaacagacagctcagtcgtgaggaaatttatacgttattacgtaagcagtctattgttcgccggcagataaaagatttagaactccagattatacaaattcaggaaaaacggagcgagctggaaaagaaaagggaagagtttcagaaaaaaagtaaatattggttgcgcaaagaagggaactatcaacgctggataatccgtcagaaaagattctatatccagcgagagatacagcaggaagaggccgagtcagaggagataatttaatgggcgatgtgtcagctgtcagttcatccgggaacattttactgccgcagcaggatgaggttggcggtttatcagaagcattaaaaaaagcggtggaaaaacataagacagaatattccggtgataaaaaagatcgcgactatggcgatgctttcgtaatgcataaagaaacggctttaccgttattactggcggcatggcgacatggcgcgccagcgaaatcagaacatcacaatggcaacgtttctggtctgcatcataacggaaaaagcgaactcaggattgctgaaaaactgttgaaagtcactgctgaaaaatctgtcggtttgatctctgcggaggccaaagtagataaatccgcagcgttgctatcgtctaaaaataggccgttagaaagcgtaagcggtaaaaaattatctgctgatttaaaagctgtggaatccgttagtgaagtaaccgataacgccacgggaatctctgacgataatatcaaggcattgcctggggataataaagccatcgcgggcgaaggcgttcgtaaagagggcgcgccgctggcgcgggatgtcgcacctgcccgaatggccgcagccaataccggtaagcctgaagataaagatcataaaaaggttaaagatgtttctcagcttccgctgcaaccaaccactatcgccgatcttagccaattaaccggcggcgatgaaaaaatgcctttagcggcgcaatcaaagccgatgatgactatttttcccactgccgatggcgtgaaaggagaggatagctcgctgacttaccgttttcagcgctggggaaatgactattccgtcaatattcaggcgcggcaagcaggggagttttcgttaataccgtcaaatacgcaggttgaacatcgtttgcatgatcaatggcaaaacggtaatccccagcgctggcacctgacgcgagacgatcaacaaaatccgcagcagcaacagcacagacagcaatctggcgaggaggatgacgcctgatgtcattgcgtgtgagacagattgatcgtcgcgaatggctattggcgcaaaccgcgacagaatgccagcgccatggccgggaagcgacgctggaatatccgacgcgacagggaatgtgggttcggttgagcgatgcagaaaaacggtggtcggcctggattaaacctggggactggcttgagcatgtctctcccgctctggctggggcggcggtttctgctggcgctgagcacctggtcgttccctggcttgctgcaacagagcgaccgtttgagttgcccgtgccgcatttgtcctgtcggcgtttatgcgtagagaaccccgtaccgggaagcgcgctgccggaagggaaattgttgcacattatgagcgatcggggcggcctgtggtttgagcatcttcctgaactgcctgcagtcgggggcggcaggccgaaaatgctgcgttggccgttgcgctttgtaatcggtagcagtgatacgcagcgttcgttgctgggccgaatcgggatcggagatgtactcctgattcgtacttcccgtgcggaagtttattgctacgcgaaaaagttaggtcatttcaaccgtgttgaagggggaattattgtggaaacgttagatattcaacatatcgaagaagaaaataatacaactgaaactgcagaaactctgcctggcttgaatcaattgcccgtcaaactggaatttgttttgtatcgtaagaacgttaccctcgccgaactcgaagccatggggcagcaacagctattatcactgccgaccaatgctgaacttaacgttgaaattatggcgaatggtgttttgctgggtaatggcgaactggtacagatgaatgacaccttaggcgttgagatccatgaatggctgagcgagtctggtaatggggaatgatatctcattaattgccttactggcattttccaccctgttgccatttattattgcgtcaggaacctgtttcgttaaattttctattgtatttgtcatggtgcgtaacgccctgggattacagcagataccttcaaatatgacgcttaacggcgtcgcattgctgctttctatgtttgttatgtggcccataatgcatgatgcctacgtctattttgaggacgaagatgtcacctttaatgatatttcatcattaagtaaacacgttgatgaaggtctggatggttatcgcgattatctgatcaaatattcagatcgcgagttagttcagttttttgaaaacgcgcaactgaagcgtcagtatggagaagagaccgagacggtaaagcgtgacaaagatgaaattgaaaaaccttcaatatttgcgttattacctgcttatgcgctgagcgaaataaaaagcgcgtttaaaattggtttttatctttatttgccctttgtcgtcgtcgacctggtggtatccagcgtgctactggcgctggggatgatgatgatgagtccggtgacgatatctacacctattaagctggtgctttttgtcgcgcttgatggctggaccttactgtctaagggattgatattacagtatatggacattgcaacatgacatcattacgagacgggatagttaaatggatgatttagtgtttgcaggtaataaggcgctctatcttgttttgatcctgtcagggtggccgacgattgtcgcaacgattatcggcctcctggtagggttattccagacggtaacgcaattacaggaacagacgctgccttttggcattaaattacttggcgtgtgtttatgcttgtttttactgtctggctggtatggcgaagttttactctcttacgggcgtcaggtgatattcctggcgttggctaaggggtaaaaaatgttttacgcgttgtactttgaaattcatcacctggttgcgtctgcggcgctagggtttgctcgcgtggcgccgatttttttcttcctgccgtttttgaatagcggggtattaagcggtgcgccgagaaacgccattatcatcctggtggcattgggagtatggccgcatgcattgaacgaggcgccgccgtttttatcggtggcgatgatcccgttagttctgcaagaagcggcggtaggcgtcatgctgggctgtctgctgtcatggcctttttgggttatgcatgcgctgggttgtattatcgataaccagcgaggggcaacgctaagtagtagtatcgatccggcaaacggtattgatacctcggaaatggctaatttcctgaatatgtttgccgctgtcgtttatttacaaaacggcggtctggtcacgatggttgacgtgttaaataaaagctatcagctatgcgatccgatgaacgagtgcacgccttcattaccgccgctattaacgtttattaatcaggtggctcaaaacgccttggttctggccagtccggtggtattagtgctgttgctgtcagaagtattcctgggtttattgtcgcgctttgctccgcaaatgaacgcttttgcgatttcactgacggtaaaaagcggtattgccgttttaattatgctgctttatttctctccggtactaccggacaatgtactgcgactctctttccaggccacagggttaagcagttggttttacgagcgaggggcgacgcatgtcctcgaataaaacagaaaaaccgactaaaaaacggctggaagactccgctaaaaaaggccagtcatttaaaagtaaagatctcattatcgcctgcctgacgctgggaggaattgcctatctggtgtcgtatggctcatttaatgagtttatggggataattaagatcattattgcggataattttgatcagagcatggctgactacagtttggccgtttttgggatagggttaaaatatctgattccatttatgctgctctgcttagtgtgttccgcattaccggcgttattacaggccggttttgtgctggcgacagaagcattaaagcctaatttatcggcgttaaacccggtagaaggggcaaaaaaactttttagtatgcgcacggttaaagatacggtcaaaaccctactgtatctctcatcctttgtggtggccgccatcatttgctggaagaaatataaggttgaaatcttttctcagctaaatggcaatattgtaggtattgccgtcatttggcgtgaacttctcctcgcattggtattaacttgccttgcttgcgcattgattgtcttattattggatgctattgcggaatatttcctgaccatgaaagatatgaaaatggataaggaagaagtgaagcgtgaaatgaaggagcaggaagggaacccagaggttaaatctaaaagacgtgaagttcatatggaaattctgtctgaacaggtgaaatctgatattgaaaactcacgcctgattgttgccaaccccacgcatattacgatcgggatttattttaaacccgaattgatgccgattccgatgatctcggtgtatgaaacgaatcagcgcgcactggccgtccgcgcctatgcggagaaggttggcgtacctgtgatcgtcgatatcaaactggcgcgcagtcttttcaaaacccatcgccgttatgatctggtgagtctggaagaaattgatgaagttttacgtcttctggtttggctggaagaggtagaaaacgcgggcaaagacgttattcagccacaagaaaacgaggtacggcattgagccgcgtaaggcagtagcgatgtattcattgggcgttttttgaatgttcactaaccaccgtcggggtttaataactgcatcagataaacgcagtcgttaagttctacaaagtcggtgacagataacaggagtaagtaatggattatcaaaataatgtcagcgaagaacgtgttgcggaaatgatttgggatgccgttagtgaaggcgccacgctaaaagacgttcatgggatccctcaagatatgatggacggtttatatgctcatgcttatgagttttataaccagggacgactggatgaagctgagacgttctttcgtttcttatgcatttatgatttttacaatcccgattacaccatgggactggcggcagtatgccaactgaaaaaacaatttcagaaagcatgtgacctttatgcagtagcgtttacgttacttaaaaatgattatcgccccgttttttttaccgggcagtgtcaattattaatgcgtaaggcagcaaaagccagacagtgttttgaacttgtcaatgaacgtactgaagatgagtctctgcgggcaaaagcgttggtctatctggaggcgctaaaaacggcggagacagagcagcacagtgaacaagaaaaggaataattatggtaaatgacgcaagtagcattagccgtagcggatatacccaaaatccgcgcctcgctgaggcggcttttgaaggcgttcgtaagaacacggactttttaaaagcggcggataaagcttttaaagatgtggtggcaacgaaagcgggcgaccttaaagccggaacaaagtccggcgagagcgctattaatacggtgggtctaaagccgcctacggacgccgcccgggaaaaactctccagcgaagggcaattgacattactgcttggcaagttaatgaccctactgggcgatgtttcgctgtctcaactggagtctcgtctggcggtatggcaggcgatgattgagtcacaaaaagagatggggattcaggtatcgaaagaattccagacggctctgggagaggctcaggaggcgacggatctctatgaagccagtatcaaaaagacggataccgccaagagtgtttatgacgctgcgaccaaaaaactgacgcaggcgcaaaataaattgcaatcgctggacccggctgaccccggctatgcacaagctgaagccgcggtagaacaggccggaaaagaagcgacagaggcgaaagaggccttagataaggccacggatgcgacggttaaagcaggcacagacgccaaagcgaaagccgagaaagcggataacattctgaccaaattccagggaacggctaatgccgcctctcagaatcaggtttcccagggtgagcaggataatctgtcaaatgtcgcccgcctcactatgctcatggccatgtttattgagattgtgggcaaaaatacggaagaaagcctgcaaaacgatcttgcgcttttcaacgccttgcaggaagggcgtcaggcggagatggaaaagaaatcggctgaattccaggaagagacgcgcaaagccgaggaaacgaaccgcattatgggatgtatcgggaaagtcctcggcgcgctgctaaccattgtcagcgttgtggccgctgtttttaccggtggggcgagtctggcgctggctgcggtgggacttgcggtaatggtggccgatgaaattgtgaaggcggcgacgggagtgtcgtttattcagcaggcgctaaacccgattatggagcatgtgctgaagccgttaatggagctgattggcaaggcgattaccaaagcgctggaaggattaggcgtcgataagaaaacggcagagatggccggcagcattgttggtgcgattgtcgccgctattgccatggtggcggtcattgtggtggtcgcagttgtcgggaaaggcgcggcggcgaaactgggtaacgcgctgagcaaaatgatgggcgaaacgattaagaagttggtgcctaacgtgctgaaacagttggcgcaaaacggcagcaaactctttacccaggggatgcaacgtattactagcggtctgggtaatgtgggtagcaagatgggcctgcaaacgaatgccttaagtaaagagctggtaggtaataccctaaataaagtggcgttgggcatggaagtcacgaataccgcagcccagtcagccggtggtgttgccgagggcgtatttattaaaaatgccagcgaggcgcttgctgattttatgctcgcccgttttgccatggatcagattcagcagtggcttaaacaatccgtagaaatatttggtgaaaaccagaaggtaacggcggaactgcaaaaagccatgtcttctgcggtacagcaaaatgcggatgcttcgcgttttattctgcgccagagtcgcgcataaaaactgccaaaataaagggagaaaaatatgttaattagtaatgtgggaataaatcccgccgcttatttaaataatcattctgttgagaatagttcacagacagcttcgcaatccgttagcgctaaagatattctgaatagtattggtattagcagcagtaaagtcagtgacctggggttgagtcctacactgagcgcgcctgcgccaggggtattaacgcaaacccccggaacgatcacgtcctttttaaaagccagtattcaaaataccgacatgaatcaggatttgaatgctctggcaaataatgtcacgactaaagcgaatgaggttgtgcaaacccagttacgcgagcagcaggcagaagtcggaaagttttttgatattagcggaatgtcttccagtgccgttgcgctgttggctgccgcgaatacgttaatgctgacgttgaaccaggctgatagcaaactgtctggtaagttgtcattagtcagttttgatgcagctaaaacgacggcaagctccatgatgcgcgaagggatgaatgcgttgtccggtagtatttcccagagcgcgcttcagttggggatcactggcgtgggcgccaaactggaatataaggggctgcagaatgaaagaggcgcgcttaaacataatgccgcgaagatcgataaactgaccactgaaagccacagtattaaaaacgtgctgaacgggcagaatagcgtcaaactcggtgctgaaggcgtcgattctctgaaatcgttaaatatgaagaaaaccggtaccgatgcgacgaaaaatcttaatgatgcgacgcttaaatctaatgccggaaccagcgccacggaaagtctgggtattaaagacagtaataaacaaatctcccctgaacatcaggctattctgtcgaaacgtcttgagtctgtcgaatccgatattcgtcttgagcagaataccatggatatgacccgaatcgatgcgcgcaagatgcagatgacgggcgatctgattatgaagaactcggtcacggtcggtggtattgcaggggcgtccgggcagtacgccgctactcaggaacgttccgagcagcaaattagccaggtgaataaccgggttgccagcaccgcatcggacgaagcccgtgaaagttcacgtaaatcgaccagcctgattcaggaaatgctgaaaacaatggagagcattaaccagtcgaaagcatccgcactcgctgctatcgcaggcaatattcgcgcttaatctgaaaggtcatctatacgccatcatgggtgtgatttaatcgcgctcctgatggcgaactggggatattatgcttaatattcaaaattattccgcttctcctcatccggggatcgttgccgaacggccgcagactccctcggcgagcgagcacgtcgagactgccgtggtaccgtctaccacagaacatcgcggtacagatatcatttcattatcgcaggcggctactaaaatccaccaggcacagcagacgctgcagtcaacgccaccgatctctgaagagaataatgacgagcgcacgctggcgcgccagcagttgaccagcagcctgaatgcgctggcgaagtccggcgtgtcattatccgcagaacaaaatgagaacctgcggagcgcgttttctgcgccgacgtcggccttatttagcgcttcgcctatggcgcagccgagaacaaccatttctgatgctgagatttgggatatggtttcccaaaatatatcggcgataggtgacagctatctgggcgtttatgaaaacgttgtcgcagtctataccgatttttatcaggccttcagtgatattctttccaaaatgggaggctggttattaccaggtaaggacggtaataccgttaagctagatgttacctcactcaaaaatgatttaaacagtttagtcaataaatataatcaaataaacagtaataccgttttatttccagcgcagtcaggcagcggcgttaaagtagccactgaagcggaagcgagacagtggctcagtgaattgaatttaccgaatagctgcctgaaatcttatggatccggttatgtcgtcaccgttgatctgacgccattacaaaaaatggttcaggatattgatggtttaggcgcgccgggaaaagactcaaaactcgaaatggataacgccaaatatcaagcctggcagtcgggttttaaagcgcaggaagaaaatatgaaaaccacattacagacgctgacgcaaaaatatagcaatgccaattcattgtacgacaacctggtaaaagtgctgagcagtacgataagtagcagcctggaaaccgccaaaagcttcctgcaaggataacagaagaggatattaataatggttacaagtgtaaggactcagccccccgtcataatgccaggtatgcagaccgagatcaaaacgcaggccacgaatcttgcggcgaatctttccgcagtcagagaaagtgccacagcgacgctgtcaggggaaattaaaggcccgcaactggaagattttcccgcgctgatcaaacaggcgagtctggatgcattgtttaaatgcgggaaagacgctgaggcgttaaaagaagtttttaccaattcaaataatgtcgccggtaagaaagcgataatggagtttgccgggctctttcgttcagcgctcaacgccaccagtgattctcctgaggcgaagacgctactgatgaaggtgggggcagagtataccgcgcaaatcataaaagatggcctgaaagaaaagtcagcttttgggccatggctgccagaaacaaagaaagcggaagcgaagctggaaaacctggaaaagcagctgttagatattatcaaaaataacactggcggtgaattaagtaaattatcgacgaatcttgttatgcaggaggtgatgccctatattgccagctgcattgaacataactttggctgtacgttagatccgttaacccgcagcaatcttacgcaccttgttgacaaagcggcggcgaaggctgttgaggcgcttgatatgtgccaccaaaaattaacgcaagagcagggtaccagcgtaggacgggaagcccggcaccttgaaatgcaaacgttgatacccctgctgctacgtaatgtttttgcacaaattcctgcagataaactgcctgaccctaaaattccggagcctgcggctggaccagtacctgatggtgggaaaaaagcagaacctacgggtattaatatcaatattaatattgatagcagtaaccatagcgtggataacagtaagcatattaacaatagccgaagccatgtcgataatagccagcgccatatcgataatagcaaccatgataatagccggaagacgattgataatagccgaacatttattgataacagccaacgcaatggcgagtcacaccattcgactaacagcagcaacgtaagtcatagtcattcgcgtgtggattcgactacgcatcaaacggagacggcacacagcgccagcacaggggcaattgaccatggcatcgcgggtaaaattgacgtcacggctcatgcgacggcagaggctgtgaccaacgcttcatccgaaagtaaagatggaaaggtggtcacgtcagaaaagggcactacgggtgaaacaacctcttttgatgaagtcgatggcgtaaccagcaagagcattatcggcaagccggtacaggccacggtgcacggcgttgatgataataaacagcaaagccagacggcagagattgtgaatgtgaagccgcttgccagtcaactggctggcgtcgagaatgttaaaaccgataccttacaatcagacacgacggtaattacaggtaataaagccggtacgaccgataatgataatagtcagacagataagactggcccattttctggtttgaagtttaagcaaaatagtttcctctcaacagtaccgagcgttacgaatatgcattcaatgcatttcgacgcccgtgagacgtttttgggtgtgatacgtaaagccctggagccagatacctccacaccgttccctgtacgcagagcgtttgacggcttgcgtgcggaaatattacccaatgacacgataaagagtgcagcgttgaaagcgcaatgtagcgatattgacaagcacccagaattgaaagcgaaaatggagactctcaaagaggtcattactcatcatccacaaaaagaaaaactggctgagattgcactgcagtttgccagagaggcggggctgaccaggctaaaaggggaaactgactatgtgttaagtaatgtgctggacggccttatcggagacggtagctggcgagctggcccggcttacgagtcatacctgaataaacctggcgtggatcgggttattactaccgttgatggcttgcacatgcagcgttaattaaccgggaaagatgcgatgaatatggatattgaagcaagagtcaaaaaagtgatcacctcttgtattgccgttgatgttgatagtatcaatggtcagacccatctggttgaggatctttacgctgactcattggatttaattgatattgtatttggtcttagtgaggagtttgacattagttgcaatgaaaacgatcttcctgatatgatgacctttgcggatatatgccgtgttgttaaaaaaagtcttgagtccagggtgtagtatttttctctcgcttgacaacaattgaataagattaattgttatgaaaatcatcacacatgtagtacccggttcaggtatggctgcaatatatgatgatattgctgacagttcgcgttttgttattaaaggcaagttacgtcatgttgaaaatgatccgaaggagctgctgatatgtgttccgatgcgtagtgaatggctattctactggattaaaggagagaaatattgcgcccggcgatgggcgcgaaaaagtatcaagacattgtgtaaccagattaaatttgaagaagcaatcttataaaagatataattcaagaggaaagtaaattgcaagcacaccaggatattatcgctaatattggtgagaaattgggtttaccgctcacttttgacgacaacaatcagtgcttattattactcgatagcgatatttttacgtctattgaagctaaagatgatatctggttattgaacggtatgattataccgttatcgcctgtttgtggcgattctatctggcggcagattatggtgattaatggtgaactggctgcgaataatgaaggtacgttagcgtatattgatgccgcagagacgttgttgcttatacatgcaattaccgatctgacaaatacttaccatattatatcgcagcttgagtcatttgtgaatcagcaggaagcgctcaaaaacatactgcaggaatatgctaaagtatgaggagagaaaattgaataatttaacgttgtcttcgttttcaaaagttggtgtgtcgaatgatgcccgactttatattgctaaggaaaatactgataaggcatatgttgcgcctgaaaaattttcgtcaaaagtattaacctggcttggaaaaatgccgttatttaaaaacactgaagtggtgcaaaaacatacggaaaatatcagagtacaggaccaaaagattttacagacatttctccatgcactaacggaaaaatatggggaaacagcggttaatgacgcactgttaatgtcccgtataaatatgaacaaaccccttacccaacgtttagcagtgcagatcacggagtgtgtaaaagctgctgacgaagggtttataaaccttattaagagcaaggataatgttggtgtcaggaatgccgctttagtcataaaaggcggcgatacaaaagtggcagaaaaaaataacgatgttggagcagaaagtaagcaacctttactcgatatcgcgctaaagggacttaaaagaacattaccgcaactggaacaaatggatggaaatagcctgcgagaaaacttccaggagatggcttcaggtaacggcccgctgcgttcattaatgacgaatttacagaatttaaataaaattccagaggctaaacaacttaatgattatgttacaacgttaacaaatattcaggtcggtgtagcccggttctcacaatggggaacctgtggaggagaggttgagaggtgggttgataaagcctctactcatgaattaacccaggctgtaaaaaaaattcacgttattgctaaagaactgaaaaatgttacagctgaacttgagaaaatagaagccggcgcgccaatgccacagacgatgagcggaccgacactgggcctggcacgatttgcggtcagcagcattccaattaatcagcaaacccaggtgaaactgagcgatggaatgcctgtgccagtgaatacgttaacttttgacggtaagcctgtggcattagccggttcgtacccaaaaaatacgccggatgcgctggaagcgcatatgaaaatgcttcttgaaaaagaatgctcgtgcctggtggtgttaacgtcggaagatcagatgcaggcaaaacaattaccaccctatttcagagggagctacacctttggcgaggtgcataccaacagccaaaaagtgagctcagccagtcagggagaagcgatagaccaatacaatatgcaactgtcctgcggggaaaagcggtatacaatcccggtattgcatgtgaaaaattggccagatcaccagccgttaccgtctacggatcagttagaatacctggcggatagggtgaaaaatagtaaccaaaatggcgcgccggggcgtagttcatcagataagcatttaccgatgattcattgtctgggcggagtgggaagaaccggaacgatggcggcggcccttgtacttaaggataatcctcatagtaatctggagcaggtacgtgcagatttccgggattcacggaacaatagaatgctggaagacgcctcacagtttgtacaactaaaagcaatgcaagcccagttgcttatgacgacggcaagctgataaaaacatagcttacttttagaactatctgaaagtaagctatttctgtataattatttgtttgccgcgatagaaagtcttttgtttttctcttctgctgacattccttttaattttctgtaattctcccaaatttttttagcataacgtttccttatatccgatcgtttcggcgacgtcccggcattataagcgccaacggcctcccagctataaccgtagattttcatcatatctgataaaatggaggcgcccacaatgacagaaatgcaggggtcctgtaacaactgtttttcactaatccccatttttttcagccttttcatatggaagctgttaatttgcatcaggccaagatcggttgaaccatctcggttatgaccaatggcgccaggtttcatcgccgattcctgctgggcgatagcgtaaagtagttcggattcaatattgaacattttttcagcctgaagccagcaatcagcccatgccgtatttatgctaagcaaccagattacgatgataaaaaaataatgcatatctcctctctcagattttaccgtaatttaatcaagcggggatcctgtttccatcttttgaaccaaatattgtcttcgtttttaaatttattccacattttctcggcaatagcttcgccgtgggcaaccagcactaacggtaataatcccggattattatctatacgctgttcactttccagaaattctcttatcgtcggtaaggcacgctcactattctgacaatattcagcgtaaagaagattaacagcaataagtcctgttatttcctgcgtggatatttctttagttaattttcgtgccagttcatgtttacctttaagcgaaagaaacataacctgcatacttaataatattggattatcctgcaggtgttgtgagcgtaattcatcgcctaaacgtatagcatcatcaataccggtatgataataggtaatccacagcttagtgatccctgcggctgcgcgcgttgggtccaattttaaacactcgttaatcgtttgtaaggcctcctccaactgaccagccatgaaaagattccagccataataatatttaatatctgcagaaatgggcgaaagtaagttagcttgtttgaatagcaaactcccgacgatgtattctgagtgaatcgtattaattagccccagtaatcctaaagcttgtggattattgtggtccagctctgtcgccttaatcgcatgttctttagctttgatcatagcgttttgtttatcaaaaatccccatttgcgccatgctgaggtagcattctgccagcgcacagtaaggcgcaatgctgtttggcgacatgttaacgcattgagtcagcaatttaagcgcttgctgtaagctatagggggtgtattgatttaactcatgcttaccgcgtaagtaaaccatagtactgtcaatcgaatttagctcgctaatctgctttgtgtcccagcgaagtccgggaatacatctgagcaaaagattcgcaattttgttttgcaagagagaagcgggttggtgttctatcaacttaatgctttcctggtgcagcaggtgataacctttaacccgaactatctcaatctgtacaatattatcattaccatcgggtatcatctgcccggagatataataatcggggcgtaattgatccatgagctcaagaatatccttaacactgcggcagttcttcgtaatggtcaccggcagcacgctcaggccaaagggcgcatactgcgataatcccttcacgatagagtaatgcagactctcggattgaacctgatcctgcatctgaaaaggaagtatcgccaatgtatgagtcgtaggttgcggcgctggcggagacaccactacgaccggacgattaaaccgatagccctgtccgtacagtgtttcaatgtaacgatgctctttatcttccgacagaatacgtcgtaaggcataaatacagcgggtaagagattcttcgttaacttccgcgtcgccccatacctggtccagtaaggtgtttttactcacaatctcgccggcggcttcgagcaggatgaccagaacggcatattcttttggcggaatattgactttcttttctgagcgtagcagggagccgtccatgttgagtatgaaatcatcaaagacgaattttttattcgatacaggaacaggattaaaatgtggcatgataatagtgtattctcttacagggtgaaaagttataataactaatacaagtcgttaggatagaatctactgtttcagtaattctgctgttagtactaacggtcaggttgagcttttattatgagcttaatgtcatattctacgggctcgggtttatatgtttttaacatttgattatttagcttatgcctgtgctttaaataactgacatgttggtaataatattgttataactaactgtgattatcgaatggacgctgccgtatatcctggtgcagagagagtcagcgccgggcatctaaatatttacatatttaacttggcctcattgcaatagagattagttttgtagctatcttactgcatttttttggggtgtaaatgctgcttattatatcttcatggttaatggtctgataattacaccatcagaaccatttttctcgaagatttccactaaatgaccattcgttgaaagtttaagagtgtaatttgtcttaggttccaaaatataaatgaaagactgtttttaatggtgcgcttatttttatatttttttgcaaaataatgatatcgtcttttctttactcccttcagttatagcgtcaaaaaggcaggagggttatgagcagtatcatcctcaggctggctccaggcattatatcgatatcaggaggaagagaggaggtatgcctggcagaaagctaacaagcgtgactgtttcggtataaaccgttcaggcaaatagttctcagagggaacggatgatgtataaatatgaataaaatgccggccttaatccacagggttaaagccggaaggagatagtgtcatctggacgaattcttacgatgtgaataaggcaatatcgttttaccagtcatcatagcgatgacaagttcacaaaaatcgtgttatataatcagccttactttaaattaccatagatatcagtataagctgtcttccggacagaacaatgatattgaatagcctcccatcctgatagagcgtgttaatgcgcagtctgaattttaaattattacaattttaataaaaatctttacttaagtgacagatacaaaaaatgttaatggttcgccatttttatgaatgtcgatggcgtagttttaaaatattttttgaaacattgaatgaagtaggacgtgctatcataaccacattttaatgctacagcattaacattatggttgcctatgcgtaaaagttttgctgcctgattcattcttgccgataagtagatgtcgctaaagctggtaccttcttctgcaagtttccgtttgagcgttgacgtactcataaatatatgatcggcaacatccgtaagcttccactgtctactgggtgacgaagatataatgttgtaaacgcgctcctttaacgttatctgagccgagctaaggatgatctcataactctccgggagtcggagaaaagcagtaagcaggaacagcagaaaataaggaattaactcttcattttcaatacaacttttgttgttacagttactgcaacctttgcttgtatccttcgtacaggagaacgccgttttcagatgttcaaatacctctcttctggcaggaaagtcaggcgtatagaagatcttctgcgctttctctgtgggtaccgccattttggtttgctgctcgtttgggataagtgcatagagagcgccaagtcgttgcgtcggtatctcgagtatatcgaaatccatgtggccattgacctcttcaagcgtcacgttaactacctgctcttttttgagcaccaacatcccaggttcgtcacagtaaatcgtatcgtgattattgctaatcgtcagtttaccgctccgaaagcaaactaaagtgaaactgcttacataaagatttttgatggtaacctgctgagtctgacttttaatttgctgccgggtatttgtcaaaagtgattttaatttctgtaagttatctgcggcaggacgctgatgactattacttacaaaggttacattttccatattatccctttgttgatgttattttaatgttccttactggtatcctactgaaaaaatctgagttgtaaatgctctttattagcgtgtgttggcaatggtctgattgttacaccaaaagaacccaaatttgggtaatttatctacagtagtttaagccccaatggggatgatggttcttttaatatgtgttgagacgcattatacagaataaattgattttatttctcacttttcattctattttcatcaggaatccctgtgtcctgtgcggtaatctgctgctatcgagaacgacagacatcgctaacagtatatatggaaacatcaaaagagaagacgataacaagcccagggccatacatagttcgattacttaacagctcactgaacggctgtgagtttccattgctgacaggccgaacactctttgtggtaggtcagagtgatgcgctcactgcttcaggtcaactccctgatatacctgccgatagcttttttatcccgctggaccatggcggagtaaattttgaaatccaggtggatacggatgcgaccgaaattatactccatgagctgaaagaaggaaattctgaatctcgttcggtgcaattaaatacgccaatacaggtcggtgaattgcttatcctgattcgcccggaaagcgagccgtgggtgcccgagcagcctgagaagttagaaacgtctgcaaaaaagaacgagccgcgttttaaaaacggaattgtagcagcactggccgggttttttatattgggaattgggactgtggggacgttatggatacttaactcgccgcagcggcaggccgcagagctcgattcgttattggggcaggagaaggagcgttttcaggtgttgccaggccgggacaaaatgctctatgtcgctgcgcaaaatgaaagagatacgttgtgggctcgtcaggttttagcgaggggcgattatgataaaaatgcgcgagtgattaacgaaaacgaagaaaataagcgtatctctatctggctggatacctattatccgcagctggcttattatcggattcatttcgatgagccgcgtaaacccgttttctggctaagccgccagcgaaacacgatgagcaagaaagagctcgaggtgttaagtcaaaagctgagagcgctaatgccttacgcggattcggttaacatcacgttgatggacgatgttaccgcagcaggccaggcggaagcggggctaaaacagcaggcgttaccttattcccgcaggaatcataaggggggcgtaacgtttgttattcagggggcgctcgatgatgtagaaatactcagagcccgtcaatttgtcgatagctattaccgcacatggggaggacgctatgtgcagtttgcgatcgaattaaaagatgactggctcaaggggcgctcatttcagtacggggcggaaggttatatcaaaatgagcccaggccattggtatttcccaagcccactttaatttaacgtaaataaggaagtcattatggcaacaccttggtcaggctatctggatgacgtctcagcaaaatttgatacgggcgttgataatctacaaacgcaggtaacagaggcgctggataaattagcagcaaaaccctccgatccggcgctactggcggcgtatcagagtaagctctcggaatataacttgtaccgtaacgcgcaatcgaacacggtaaaagtctttaaggatattgatgctgccattattcagaacttccgttaatcagttataaggtggattatgtcgattgcaactattgtccctgagaatgccgttatagggcaggcggtcaatatcaggtctatggaaacggacattgtctcgctggatgaccggctactccaggctttttctggttcggcgattgccacggctgtggataaacagacgattaccaacaggattgaggaccctaatctggtgacggatcctaaagagctggctatttcgcaagagatgatttcagattataacctgtatgtttctatggtcagtacccttactcgtaaaggagtcggggctgttgaaacgctattacgctcatgattcgtcgatatctatatacttttctgctggtaatgacccttgccggctgtaaggataaggatcttttaaaaggactggaccaggaacaggctaatgaggtcattgccgttctgcaaatgcacaatatagaggcgaataaaattgatagcggaaaattgggctatagcattaccgttgctgagcctgattttaccgctgcggtgtactggattaaaacttatcagcttcctccccggccacgggtggaaatagcgcagatgttcccggcggattcgctggtatcgtctccgcgagctgaaaaggccaggttatattcggctattgaacagcgactggaacagtcattacagacgatggagggcgtgctctccgccagggtccatattagttatgatattgatgctggtgaaaatggccgcccgccaaaacctgttcatctgtcggcattagccgtatatgaacgaggttcgccgcttgcgcatcagatcagcgatatcaagcgtttcttaaagaatagttttgccgatgtggattatgacaacatttctgttgtgttgtcagaacgttctgatgcccaattacaggctcccggcacaccagtaaaacgtaattcttttgcaaccagttggattgttttgattattttgttatccgtgatgtcagcaggctttggcgtctggtattacaaaaaccattatgcccgcaataagaaaggcataacggctgatgataaggcgaaatcgtcaaatgaataggcagccattacccattatctggcaaagaatcatttttgatccgttatcgtatatccatcctcagcggttgcagatagcgccggaaatgattgtcagacccgccgccagggcggcggcaaatgagttaatactggcggcatggcggcttaagaacggagaaaaggagtgtattcaaaactcactgacgcagctgtggctgcgtcagtggcgccgactgccgcaagtagcgtatttactcggttgccataaactgagagccgatctggcaaggcagggagccttgcttggcctgccggattgggcgcaagcatttttggcaatgcatcagggaacaagtttatctgtctgcaataaggcgccgaatcaccggtttttacttagcgtcgggtatgcacagttaaatgccctaaatgaatttttacctgaatctttagcacagcgttttcctttgctttttcctccatttattgaggaggcattgaagcaggatgctgtagaaatgtcaattttgctactggccttacaatatgctcaaaaatatcccaataccgtccccgctttcgcctgttgaggggatactgataaagcgtaaaacgctggaacgttatttctctattgaaagattagaacagcaggcgcatcaacgggctaagcgtattttgcgagaggcggaagaagaggcaaagaccttgcggatgtacgcctatcaggaaggttacgagcagggaatgatagacgcgttacagcaggtcgccgcttatcttactgataatcagacaatggcctggaagtggatggaaaaaatacagatttatgcccgcgagttattttcagctgcggtcgaccatcccgaaacgcttttaaccgtcctggatgagtggctaagggatttcgataagcctgaggggcaactttttttaacactgccagttaatgcgaaaaaagatcaccaaaaactgatggtgttgcttatggagaactggccaggcacttttaatcttaaatatcaccaggaacagcgctttatcatgagttgcggcgatcagatcgcagaattttcacctgaacaatttgttgaaacggcagtaggcgtcattaagcatcatcttgatgaacttccacaagactgccggacaatttctgataacgccattaacgcacttattgatgaatggaagacaaaaacgcaagcggaggttataaggtgataccgggtacgattccgacttcttatttggtcccgacagcagatactgaagcgacgggtgtggtttcgttgagtgccagggccgctatgctgaataatatggatagcgcgcctttaagcaatggcggcgacgttgatctttatgatgcattctaccaacgacttttggcgcttcctgagtcagcctcttctgaaacgcttaaagatagcatttatcaagagatgaatgccttcaaagatcctaacagtggtgattcggcttttgtttcttttgagcagcaaacggctatgctacaaaacatgttagcaaaagttgaaccgggcacccatttatatgaggctttaaacggggtattagttggttcaatgaacgcacagtcacaaatgacctcctggatgcaggagattattttatcgggcggggaaaacaaagaggcaattgactggtgaacccccattgctggcgatttgtgataaggtatggtgtatatatcagcaaataatgcagaaaatgcaccatgccagtgtgtctatcttattgatgtatatggattattaagatgtctgccagccgttttattctgaaatgattatattaatattgtaagctttcattacaaaattgtgcataaagtttgtaagggtatctttttgtgacgaaatgaacgcgcgttggaatgtaattattggctataataataaaaaaatcggatttaaatcatctctgtgagttttaattatttgtttataagaatataacgattttgagttccttatagcacacaggataaaatatggtattgccttcaatgaataaatcagttgaggccattagcaataatcaccttcaacagccgaacaaatttccattaataaatggattagctgacgtaagagactattatgtcgcaaactgcttattgtttaaacttaataaaggcagtttgcgaattgaaaacgaatttggggagttcatcgaacgatctgcgccgtgtttatttttattggaaaaagatcaaacaatcacgcttagtatgagcgaaatagaagggcatattgatttttcttcactggaagtttcctatgacttaatgcaaaaattctacaaagttttttacagtacaagaaactataatgatcgagagctatcattaaaaacgaaaccaaagtatttttttcatgcggacttgttgccagggatgagtgatacttttgactctattttgcatggtgtggcatgtccacgggtttgtagtaatgtgagtattgatgatcatgattattcatatttctcattgatgtatcttatatcggcatttgtacgtaagcccggtgggtttgatttccttgagcgagcaataaaaattacgacaaaagagaaagtttataacattattatcagcgatctcacccgcaaatggtcacaggctgaggtggcaggaaagctgtttatgagcgtatcaagtctgaagcgaaaactggccgctgaagaggtgagttttagtaaaatatacctggatgctcgtatgaatcaggctataaaattattacgtatgggggctggaaatatttcacaagtcgcgacgatgtgtggctatgatacgccttcttattttatcgctatttttaaacggcattttaagattacaccgcttagctttatgcgtacaatgaaccattgatttgtgaaattattttaaacgttactatctgtttgcgttacagataccaaatatttttttaatcgtagtgtatatttcagtatcgctacaccagtgatatgtagttaatgaaagggaatcgaaagcgttcattgtcagacatacatggccaccaggcgccgggcaatcgttgtactctaagagattacagtaaagtaaaacagcaaatttaatcattatcagatttgtaaaaggaattcatttcggtaacgacattgcgcatgtaataacgtatctggtcttattacctttgtagtaagaaggcgttatctacttgcgcagtagtcgcccaggaagaaaaatcattaccgaagctgtggtcagttttcaaaaaaggataaataaatgagaaatgtaattatatacggtattaactggactaattgttatgccctacagtctatttttaagcaaaaatatccggaaaagtgcgttaaaacgtgtaactcattaactgcacttttgcattccctatccgatatgccggacgccgggctgattttagctttgaacccgcatgagcatgtttatctttttcatgcgttgctgacgcggttgcagaaccgtaaagttttggtagtggcagatcgcttgtattatatcgatcgctgtgtgctgcaatattttggcgttatggattatgttttaaaagacgaactatcctgcgctatccgctcggagcgagagaagctccgtcttccggaagcctggctgcgtttctgccacaggccacaaaagaaaaccgtggctgctacgtatgcttttaatgccggcgagacgccggaagaggtattgtttaatatcaatcaatacgcctggtggaatctacctcccggtgtcacgcaggcgaaatatgcgctgctgatattattatcctccggacatccggcaattgaactggcgaaaaaatttggtctgggaacaaaaaccgtcagtatttatcgtaagaaggttatgtatcgtttggggatggactcttcaccgctatcgctgttccggggactgaaactagacgcgcatttacagcgcactgcttttgcacataaccctgctgtacctgacgataattgcgcgttaccgattgcggtaggaatgaattaaaatattttttatcatttatgaccatgtgttgagcttttattataaaaaagattttttgagtagtaattcttatatataatcatccggaggtggttggtagcctggctcaatcattgaggcatatttttgcaggcaatatattgaatctgaaaagttaaagatgatattttcggtgcaggagctatcatgtggagggaaaagtatgctaagtcctacgactcgtaatatgggggcgagtttatcgcctcagcctgacgtcagcggggagctaaacaccgaagcattgacctgtattgttgagcgtctggaaagtgaaattatagatggcagctggattcatatcagttacgaggaaaccgatctcgaaatgatgccttttcttgttgcacaggccaataagaagtatccagagttaaatcttaaatttgttatgtcagtccatgagcttgtttcctctataaaggagaccagaatggaaggcgttgaatctgcccgatttctcgtaaatatgggaagttcaggtatccatatttcagtcgtcgattttagagttatggacggaaagacatcggtgattttgttcgaaccagcagcgtgtagcgcttttggacctgcactggcgttgaggaccaaagcagctcttgaacgtgaacaactgcctgattgttattttgctatggtcgagctggacattcaacgaagctcttctgaatgcggtatttttagcctggcgctcgccaaaaaacttcagcttgaatttatgaacttagtaaaaattcatgaagataatatttgtgaacgtctgtgtggtgaagaaccttttctcccgtccgataaagcagaccgctatctgccggtgagtttttacaaacatactcaaggcgcacaacgattaaatgaatatgtggaggccaatccggcggcgggaagcagtatagtaaacaaaaagaatgaaacgctttatgagcgattcgataacaatgccgttatgctaaacgataaaaaactctctatatccgctcataaaaaaaggatagctgaatataagtctttacttaaaccgtaatgaaattataaggttgcctgccagaggaaatccttccagc

SEQ ID NO: 2 - DNA, 25440 bp, Unknown
  Salmonella pathogenicity island-2
ttttgtcgatgatgagcaatactgcgtggcgtaaggctcatcaaaatatgaccaatgcttaataccatcggacgcccctggttaatactctattaacctcattcttcgggcacagttaagtaactctgtcactttatgaacctgtagctttctcatcatattcatccggtgtgtttcgacggtttttatactgatatgtagcttttcgctgatcccatgattggtatacccctcgtcaataagtttaagaacctgacgctcgcgcaaagtaagcagttgatgattggtcgtgtcagcgtttaattcagccaggatagcttcccgattcaacgttgggtcaatgtaacgcttgtttactgctactgtttgcaatgccgctaacagaacttgctgactactgctttttaaaacatagccattagcacctgcggctaaagttttaatggtcatatactcttgttggtatgctgtgtaaaccagaatattcattgctggccaacgctgatgtaattgaggaatgatatccaggccattgatgccaggtagactaagatcaaggataagtatgtcaggctcgtatgcacaacaggcattataaacctcaagaccatttttaacatgctctacaattttaaaatgaggccagggtaataaggcattcataatgccgttaatgatgatttcatgatcgtctactaataagatcttatattctttcattttgctgccctcgcgaaaattaagataatattaagtaatggtgtagtttttgaagatcatacgtattttctggcgtaagtcggttagttcctccagcgcgatgattttccccatttttacgcgattctcaatgtctatgacatagcataccaattcagtctgccctatttgacctaaacagccttttaatgtgtgaattaactgatcgattttttctccagccgatacggcattttcaatatcagccagcaagaggtccagtgattggaaaatcttgctattaatgaccatatcatctgtcgccagtagcgctgagcagcgactcggatcctgctcctgtagctctatatttcgtaaaagttggtattctgcggcaatactgatgtagcgagctaaggtagccaatgtcactggttttgtaatgtaatgatgaatcccattttttttacaacgatgaatatcttctgtcgctacgctagcggatagtgccacaaacatgcagtcaggatctaaattattcggctcatcatgccataatcgtacacattcaataccatctatttctggcattctaatgtcaatcagtactaaatcgaatcgctgctgttgtgataaagtcagagcctcgttactactggcggcaatagtgacgtgttggcccaggctgacaagcattttgccgatgatatcccgattaatatcggcatcatcaaccaaaagaatctgcaactgccagggtggtaacaaattatttattactggcatatttggtgtacacaatattaactgttgcgccaggtcgtagagttttccggagaaatacaaaagctctgcgttgagaagcgcattttgctggtggggtggttcaccgcgtattccccagcaagccagttgccgatgcaggcagaacggcgctgacagcgtccctttaattggttgaggcggctggtattcttgtaagggtaatactagcgagacacaggttccaaccccggggacactttttagtgtcagattaccgcccatcattttagccaggcttgacgcaatagtcagtccaattcctgtaccttgcgaatttgtgtctgcttgataaaaagcagtaaagatttgagactgctgctgtatttcaatccctttaccgctatcgctaaccagaaatattaattgttcctcatgacgcttgaccgtcagacgtatccctccggtttcggtaaattttaccgcgttcccgagtaaattaaccaaaatttgccgtaaacggatactgtcggtatgaaaatagagagggacatgttgaccgacaaaagtacgtaatgacagttttttgctttgcgctggcccctggatggtttgcattgcctggtccagtaacggcagtaacgctgtttcttccatatgtaatgtgaaatgaccagactcgatgcgtgaaaaatccagcagattattaataatagctaacaaagacagtgtacaatttctggcggtatcagctaatccttgttgctctatgtttaaaggggtggtttgtaataattcaattgcaccgagtacgccattcatcggagtacgtaactcatgacttattaccgtaagatgaatgcttttacgtttgttagctcgctcagcgcgtttttttgcttcatttagcgcctgggtgcgctctgcgactttgttttccagattgtcgtattggacttgtagagtatcaagcagttggttaaaagcaccggcaatactatctaattcatccagtcgttgtgctggtaaacgtgtgctcagcggtgcagttgcggttttattaatgacatcgacaaaacgccataacggtttggccagtgagcgatgtagtaaccagcaaaaagccgacgtcatcaacaccaatgctgttaatgtaaaggggatttgttgaaggataatttttaagatgcgattatgtagattaccgtatgggtacagcgtaaccagactccatccggggccatgcaaggttgtgcgtaatatcagaaatccgggaatttgctgccatccatcatgcagcgttacattttctaactgtgtacgtattttttgcgggatgtatgaaaacggcaataagtggttgttttgatccagccatactcgaatactatcatctaatggcaggtggctcttagtaatgagatcgggaagtttaaccgtcacctcaaaaaatacgccttgctgatcggcaaccgcaacggaagcgtgccatcctttgccgtttatgtattctggttcactccagtaaaacccggcatgggttgggtataaaggaaagctttttcgcgttaaaggctgtagagttgaataatctgaagggttatcagtagataataacgaaatctcatttttatgattaagaataaaactatcgcgacgaaagctattttcatcgatatcagaggactgcagaaagagacggtgcttctctccgtttagcgtcggcgtgcaatttgaaggaccgacagatagatgccggctcacctcagggaaaatatcgttatgatgaatctcagtcgctaatgagcattgatacattaaatttttagcgtcacgttcagcttcttcaaaccgttgattgcttagtacaatattcatctcggatagaacggataaatcctctattatatgctgccgtttctgaaccattgatatataagctgcggtaagcacagatagcagccaaataattattgttgttaataaaaataaaaaagttagcctgattactaaagatgtttgcagcgtattcttgagattgagcaaattcataatgcttccctccagttgcctgttgcaaaatctttggcacttgatcactatcgcagtacatatagtttcatcagaagattaatcgatggtgttatcattaggaagataaatttcttcatatataacccagtcgatgactacaattactttttaataagatggcgatgtaaaaacatcgtaacagtttatttaataaataatttttcaaattgtaagtttttatgtcaatgctgaaaatgtaattgtgaatttatcggaaaatccgaatgatagaatcgcctgtgacaaggtatatgtagacagcatcctgatattgtacaagaagagtatagtcgaaataaatgtgaatcaggctttttacggatgtggttgtgagcgaatttgatagaaactcccatttatgtctgaggagggattcatgctggcagttttaaaaggcattccattaattcaggatatcagggccgaaggtaatagccgatcctggataatgactattgatgggcatcctgccagaggagaaattttctcagaagcattttctatttctttgttcttaaatgacctggaaagcttacctaagccttgtcttgcctatgtgacactactgcttgcagcacacccggacgtccatgattatgctatacagctcacagcggatgggggatggttaaacggttattataccacaagtagtagctctgagcttattgctattgagatagaaaaacacctggctttaacttgcattttaaaaaatgtaatacgcaatcaccataaactttattcgggtggggtataaaatggtagtaaataaacgtttaatcttaattttactatttatactcaatacagcaaagagtgatgagttatcatggaaaggtaatgacttcaccctttatgccagacaaatgccattagcagaggttttacatctgctctcagagaactatgatacggctattactattagcccattgataacagctacatttagtggaaaaattccgcctggaccaccggtcgatattttgaataacctggcagcacaatatgatttgcttacctggtttgatggcagcatgttatatgtatatcctgcatcgttattaaaacatcaggttatcactttcaatattttatctactggacggttcattcattacttacgcagccagaatatcctttcatcaccgggatgcgaggttaaagaaattaccggtaccaaagctgtggaggtgagcggtgttcccagctgcctgactcgtattagtcaattagcttcagtgctggataatgcgttaatcaaacgaaaagacagtgcggtgagtgtaagtatatacacgcttaagtatgccactgcgatggatacccagtaccaatatcgcgatcagtccgtcgtggttccaggggtcgttagtgtattgcgtgagatgagtaaaaccagcgtcccgacgtcatcgacgaacaatggttcacccgctacacaggcattgcccatgtttgctgccgacccacgccagaatgcagtgatcgttcgtgattatgcggccaatatggccgggtatcggaaactcatcacagaattagatcaacgccagcagatgatagagatttcggtgaaaattatcgatgttaatgctggagatattaaccagttaggcatcgactggggaacggcagtgtcgctgggtggcaagaaaattgcgttcaatacaggtttgaatgacggtggtgctagtggtttttcaacggtaatcagcgatacctcaaactttatggtgcgtctgaatgccctggaaaaaagctctcaggcttatgtactttcccagccatctgtggtgactttaaataatatccaggctgtgctggataaaaatattactttctataccaaactgcagggagaaaaagtggctaaacttgaatccatcactacgggttctttgttacgcgttacacctcgcttgttaaatgacaatggcacgcaaaaaataatgcttaatcttaatattcaggatggacaacaaagtgatacgcaaagcgaaacagacccgctgcccgaagtgcaaaattctgaaattgcttcgcaagccacattattggccgggcaaagtctattgctgggagggtttaaacaaggtaaacaaatccactcgcaaaacaaaatccctttattgggcgatattcctgttgtaggtcatttgtttcgcaatgatacgactcaagtacatagtgtaatcaggctttttttgattaaagcctcagtagtaaataatggcatatctcatggttaatccaaagagttcctggaaaatacgttttttaggtcacgttttacaaggccgggaagtatggctgaatgaaggtaacctgtcactgggggagaagggatgcgatatttgtattccgctggctataaatgaaaaaattattctgagagaacaggcagatagtttatttgttgatgccgggaaagccagagttagagttaatggccgcagatttaatccaaataagccgctaccatccagtggggttttgcaggttgcgggagtggctatcgcgtttggtaaacaggattgtgaacttgctgattatcaaatacccgtttccagatcagggtactggtggttggctggcgtattcttgattttcatcggtggaatgggtgtcctgttaagtattagtggtcagcctgaaacggtaaatgacttacctttgcgggttaagtttttattagacaaaagcaatattcattatgtgcgggcgcaatggaaagaagatggcagcctgcagttgtccggttattgctcgtcaagcgaacagatgcaaaaggtgagagcgactctcgaatcatggggggtcatgtatcgggatggtgtaatctgtgatgacttattggtacgagaagtgcaggatgttttgataaaaatgggttacccgcatgctgaagtatccagcgaagggccggggagcgtgttaattcatgatgatatacaaatggatcagcaatggcgcaaggttcaaccattacttgcagatattcccgggttattgcactggcagattagtcactctcatcagtctcagggggatgatattatttctgcgataatagagaacggtttagtggggcttgtcaatgttacgccaatgcggcgctcttttgttatcagtggtgtactggatgaatctcatcaacgcattttgcaagaaacgttagcagcattaaagaaaaaggatcccgctctttctttaatttatcaggatattgcgccttcccatgatgaaagcaagtatctgcctgcgccagtggctggctttgtacagagtcgccatggtaattacttattactgacgaataaagagcgtttacgtgtaggggcattgttacccaatgggggagaaattgtccatctgagtgccgatgtggtaacgattaaacattatgatactttgattaactatccattagattttaagtgagtggaaaatgacaactttgacccggttagaagatttgctgcttcattcgcgtgaagaggccaaaggcataattttacaattaagggctgcccggaaacagttagaagagaacaacggcaagttacaggatccgcagcaatatcagcaaaacaccttattgcttgaagcgatcgagcaggccgaaaatatcatcaacattatttattatcgttaccataacagcgcacttgtagtgagtgagcaagagtaaagtaaaaatatcttagagcctatcccaccaggcgttaattggcgcagccagtttggacacggatagcgcgcaaaaaccgcagcgtacacgtagtacgtgaggtttgactcgctacgctcgcccttcgggccgccgctagcggcgttcaaaacgctaacgcgttttggcgagcactgcccaggttcaaaatggcaagtaaaatagccctaatgggataggctcttagttagcacgttaattatctatcgtgtatatggaggggaatgatgataaagaaaaaggctgcgtttagtgaatatcgtgatttagagcaaagttacatgcagctaaatcactgtcttaaaaaatttcaccaaatccgggctaaggtgagtcaacagcttgctgaaagggcagagagccccaaaaatagcagagagacagagagtattcttcataacctatttccacaaggcgttgccggggttaaccaggaggccgagaaggatttaaagaaaatagtaagtttgtttaaacaacttgaagtacgactgaaacaacttaatgctcaagccccggtggagataccgtcaggaaaaacaaaaaggtaaagcataatgtcttcaggaaacatcttatggggaagtcaaaaccctattgtgtttaaaaatagcttcggcgtcagcaacgctgataccgggagccaggatgacttatcccagcaaaatccgtttgccgaagggtatggtgttttgcttattctccttatggttattcaggctatcgcaaataataaatttattgaagtccagaagaacgctgaacgtgccagaaatacccaggaaaagtcaaatgagatggatgaggtgattgctaaagcagccaaaggggatgctaaaaccaaagaggaggtgcctgaggatgtaattaaatacatgcgtgataatggtattctcatcgatggtatgaccattgatgattatatggctaaatatggcgatcatgggaagctggataaaggtggcctacaggcgatcaaagcggctttggataatgacgccaaccggaataccgatcttatgagtcaggggcagataacaattcaaaaaatgtctcaggagcttaacgctgtccttacccaactgacagggcttatcagtaagtggggggaaatttccagtatgatagcgcagaaaacgtactcatgaaaaaagacccgaccctacaacaggcacatgacacgatgcggtttttccggcgtggcggctcgctgcgtatgttgttggatgacgatgttacacagccgcttaatactctgtatcgctatgccacgcagcttatggaggtaaaagaattcgccggcgcagcgcgactttttcaattgctgacgatatatgatgcctggtcatttgactactggtttcggttaggggaatgctgccaggctcaaaaacattggggggaagcgatatacgcttatggacgcgcggcacaaattaagattgatgcgccgcaggcgccatgggccgcagcggaatgctatctcgcgtgtgataacgtctgttatgcaatcaaagcgttaaaggccgtggtgcgtatttgcggcgaggtcagtgaacatcaaattctccgacagcgtgcagaaaagatgttacagcaactttctgacaggagctaaaaatgaatcgaattcacagtaatagcgacagcgccgcaggagtaaccgccttaacacatcatcacttaagcaatgtcagttgcgtttcctcgggttcgctgggaaagcgccagcatcgtgtgaattctacttttggcgatggcaacgccgcgtgtctgctatccgggaaaattagtcttcaggaggcaagcaatgcgttgaagcaactgcttgatgccgtacccggaaatcataagcgtccatcattgcctgactttttgcagaccaatcccgcggttttatcaatgatgatgacgtcattaatactcaacgtctttggtaataacgctcaatcgttatgccaacagcttgagcgggcaactgaggtgcaaaatgcattacgtaataagcaggtaaaggagtatcaggagcagatccagaaagcgatagagcaggaggataaagcgcgtaaagcgggtatttttggcgctatttttgactggattaccggcatatttgaaaccgtgattggcgccttaaaagttgtggaaggttttctgtccggaaatcccgcagaaatggctagcggcgtagcttatatggccgcaggttgtgcaggaatggttaaagccggagccgaaacggcaatgatgtgcggtgctgaccacgatacctgtcaggcaattattgacgtgacaagtaagattcaatttggttgtgaagccgtcgcgctggcactggatgttttccagattggccgtgcttttatggcgacgagaggtttatctggcgcagctgcaaaagtgcttgactccggttttggcgaggaagtggttgagcgtatggtaggtgcaggggaagcagaaatagaggagttggctgaaaagtttggcgaagaagtgagcgaaagtttttccaaacaatttgagccgcttgaacgtgaaatggctatggcgaatgagatggcagaggaggctgccgagttttctcgtaacgtagaaaataatatgacgcgaagcgcgggaaaaagctttacgaaagagggggtgaaagccatggcaaaagaagcggcaaaagaagccctggaaaaatgtgtgcaagaaggtggaaagttcctgttaaaaaaattccgtaataaagttctcttcaatatgttcaaaaaaatcctgtatgccttactgagggattgttcatttaaaggcttacaggctatcagatgtgcaaccgagggcgccagtcagatgaatactggcatggttaacacagaaaaagcgaagatcgaaaagaaaatagagcaattaataactcagcaacggtttctggatttcataatgcaacaaacagaaaaccagaaaaagatagaacaaaaacgcttagaggagctttataaggggagcggtgccgcgcttagagatgtattagataccattgatcactatagtagcgttcaggcgagaatagctggctatcgcgcttaatctgaggataaaaatatggaagcgagtaacgtagcactggtattaccagcgccttccttgttaacaccttcttccactccatctccctccggggagggaatgggtactgaatcaatgcttctgttatttgatgatatctggatgaagctaatggagcttgccaaaaagctgcgcgatatcatgcgcagctataacgtagaaaaacaacggctggcctgggaactgcaagtcaatgttttacagacgcaaatgaaaacaattgatgaagcgtttagagcatcaatgattactgcgggtggcgcaatgttgtcgggtgtactgacgataggattaggggccgtaggcggggaaaccggtcttatagcgggtcaagccgtaggccacacagctgggggcgtcatgggcctgggggctggtgtagcgcaacgtcaaagtgatcaagataaagcgattgccgacctgcaacaaaatggggcccaatcttataataaatccctgacggaaattatggagaaagcaactgaaattatgcagcaaatcatcggcgtggggtcgtcactggtcacggttcttgctgaaatactccgggcattaacgaggtaaacatggtgcaagaaatagagcaatggttacgtcggcatcaggtgtttactgagcctgcatatttaggggagaccgccatattacttgggcagcagtttatattatcgccttacctggtgatctatcgtattgaggcaaaagaaatgattatttgtgagttcaggcgcctgacgcccgggcaacctcgaccacagcaattgtttcacttactgggacttttacgcgggatatttgtgcatcacccgcagttaacatgtttaaagatgttgataatcaccgacgttctggatgaaaaaaaagccatgctacgcaggaaattattgcgcatcctgacagtaatgggagcgacctttacacagcttgatggcgataactggacagttttatccgccgagcatcttatccagcgacgtttttaaatgaccttcctgacgtaaatcattatcacgtgaaaataacaatcaataggtatgatgatgaaagaagatcagaaaaataaaatacccgaagacattctgaaacagctattatccgttgatccggaaaccgtttatgccagtggttacgcctcatggcaggagggggattattcgcgcgccgtaatcgattttagttggctggtgatggcccagccatggagttggcgtgcccatattgcattggctggcacctggatgatgcttaaagaatacacgacggccattaatttctatggacatgccttgatgctggatgccagccatccagaaccggtttaccaaacgggcgtctgtctcaaaatgatgggggaacccgggttggcgagagaggcttttcaaaccgcaatcaagatgagttatgcggatgcctcatggagtgagattcgccagaatgcgcaaataatggttgatactcttattgcttaaataacagaacgaaatatgaaaattcatattccgtcagcggcaagtaatatagtcgatggtaatagtcctccttccgatatacaagcgaaggaggtatcgtttcctccccctgaaattccagcgcctggcacccccgcagcccctgtgctgcttacgcctgaacaaataaggcagcagagggattatgcgatacattttatgcaatacactattcgtgcgctgggtgcgacagtcgtgtttgggttatcggttgctgcagcggtaatttctggcggggcaggattacccattgctattcttgcgggggcggcgctcgtgattgctattggggatgcttgctgtgcgtatcataattatcaatcgatatgtcagcaaaaggagccattacaaaccgccagtgatagcgttgctcttgtggtcagtgcgctggccttaaaatgtggggcaagtcttaactgcgctaacacccttgctaattgtctttctttattaatacgttcaggaatcgctatttctatgttggttttacccctacagtttccactgcccgcggctgaaaatattgcggcctctttggacatggggagtgtaattacctccgttagcctgacggcgataggtgcggtactggattattgccttgcccgcccctctggcgacgatcaggaaaattctgttgatgaacttcatgccgatcccagtgtgttattggcggaacaaatggcagcgctctgtcaatctgctactacacctgcattaatggacagttctgatcatacatctcggggagaaccatgaaacctgttagcccaaatgctcaggtaggagggcaacgtcctgttaacgcgcctgaggaatcacctccatgtccttcattgccacatccggaaaccaatatggagagtggtagaataggacctcaacaaggaaaagagcgggtattggccggacttgcgaaacgagtgatagagtgttttccaaaagaaatttttagttggcaaacggttattttgggcggacagattttatgctgttccgctggaatagcattaacagtgctaagtggtggaggcgcgccgctcgtagccctggcagggattggccttgctattgccatcgcggatgtcgcctgtcttatctaccatcataaacatcatttgcctatggctcacgacagtataggcaatgccgttttttatattgctaattgtttcgccaatcaacgcaaaagtatggcgattgctaaagccgtctccctgggcggtagattagccttaaccgcgacggtaatgactcattcatactggagtggtagtttgggactacagcctcatttattagagcgtcttaatgatattacctatggactaatgagttttactcgcttcggtatggatgggatggcaatgaccggtatgcaggtcagcagcccattatatcgtttgctggctcaggtaacgccagaacaacgtgcgccggagtaatcgttttcaggtatataccggatgttcattgctttctaaattttgctatgttgccagtatccttacgatgtatttattttaaggaaaagcattatggatattgcacaattagtggatatgctctcccacatggcgcaccaggcaggccaggccattaatgacaaaatgaatggtaatgatttgctcaacccagaatcgatgattaaagcgcaatttgccttacagcagtattctacatttattaattacgaaagttcactgatcaaaatgatcaaggatatgcttagtggaatcattgctaaaatctgaagttattagcgacgatgttcgacggttgctgctggaaatcatgtttgcgggcgttaaccatagcctgatttcccaggtacatgcgatgttaccagcgctaacggttattgttccggataaaaaattacagttggtatgtctggcattattgttggcgggtttaaatgagccgctaaaagccgcgaaaattttatcggatatagatttgccagaggctatggcgctgcgtctgttatttcctgcaccaaatgaggggtttgaaaattgaatatttctgatatgagcgtagtgcctgtaagcactcaatcttatgtaaagtcctctgcagaaccgagccaggagcaaattaatttttttgaacaattgctgaaagatgaagcatccaccagtaacgccagtgctttattaccgcaggttatgttgaccagacaaatggattatatgcagttaacggtaggcgtcgattatcttgccagaatatcaggcgcagcatcgcaagcgcttaataagctggataacatggcatgaaggttcatcgtatagtatttcttactgtccttacgttctttcttacggcatgtgatgtggatctttatcgctcattgccagaagatgaagcgaatcaaatgctggcattacttatgcagcatcatattgatgcggaaaaaaaacaggaagaggatggtgtaaccttacgtgtcgagcagtcgcagtttattaatgcggttgagctacttagacttaacggttatccgcataggcagtttacaacggcggataagatgtttccggctaatcagttagtggtatcaccccaggaagaacagcagaagattaattttttaaaagaacaaagaattgaaggaatgctgagtcagatggagggcgtgattaatgcaaaagtgaccattgcgctaccgacttatgatgagggaagtaacgcttctccgagctcagttgccgtatttataaaatattcacctcaggtcaatatggaggcctttcgggtaaaaattaaagatttaatagagatgtcaatccctgggttgcaatacagtaagattagtatcttgatgcagcctgctgaattcagaatggtagctgacgtacccgcgagacaaacattctggattatggacgttatcaacgccaataaagggaaggtggtgaagtggttgatgaaatacccttatccgttgatgttatcgttgacaggactgttattaggagtgggcatcctgatcggctatttttgcctgagacgccgtttttgagccgacctgatcccgaggtgttgcaactttatcgttatttctggcaacctgctcgttacgctgtaccggaatggctggataagctgggctttcatctttcaaactgctggcgttatggcgatcggcccgagttggatcgtcttcttgacagagcgttaaatagactaagaggaagctctgttattccagcctgtttaaatgacaggcaaaaacggcaggttcgtcttgcgccgcgtatatcggcatttgcctttgggctgggattattcaaactcaggtgtagtgactattttatgctaccagagtatcggcaattgcttctacagtggtttagcgaggatgagatctggcagctatatggttggttggggcaaagagatggcaaattacttcctccgcaagtgatgcaacaaactgcattgcagatcggtaccgccattcttaatcgggaagcgcatgacgatgcggttttacatgcgctattagtattattaccccctccgcagcgtatactttggccgaagacttctcttaccgagattatcttcatggagcatttgctatgagttttacttcacttcctctgacggaaattaaccataagctacccgctcgaaatattattgagtcacagtggataacattacaattaactttatttgcgcaagagcaacaagctaagagagtttcacatgctattgtgagctccgcttaccgtaaggctgaaaaaatcatccgagacgcctatcgttatcagcgtgaacagaaagttgagcagcaacaagaactagcgtgcttgcgtaaaaatacgctggaaaaaatggaagtggaatggctggaacagcatgtaaaacatttacaagacgatgaaaatcaatttcgttcattggtcgatcacgcagcgcatcatattaaaaatagtatagaacaggttctgttggcctggttcgaccaacagtcggtagacagtgttatgtgccatcgtctggcacgccaggccacggctatggcggaagagggagcgctttatttgcgtattcatcctgaaaaagaggcattgatgcgagaaacttttggcaagcggtttacgttgattatcgagcctggtttctctcccgatcaggctgaactttcctcaacacgatatgccgttgaattttcactttctcgtcatttcaacgcgttactgaaatggttacgtaatggtgaagataaaagaggtagcgatgaatattaaaattaatgagataaaaatgacgccccctacagcatttacccctggccaggttatagaggaacaagaggttatttcgccttcaatgttagctctccaggagttacaggaaacgacgggggcagcgctctatgagacgatggaagaaataggaatggcgctgagtggtaaactgcgcgaaaattataaattcactgatgctgagaaactggagcgcagacagcaggctttgctgcgtttgataaaacaaatacaggaggataatggggcaacgttgcgtccgcttaccgaagagaatagtgatcctgatttacagaatgcgtatcaaattatcgctcttgcaatggcgcttactgccggcgggttgtcaaaaaagaaaaaacgcgatttgcaatcgcaactggatacgcttacagcggaggagggatgggaacttgccgtttttagtttactggaacttggcgaagtggataccgctacgctgtcctctctgaagcgttttatgcaacaggcgatagacaacgatgaaatgcccttatcgcagtggttcagacgcgtggcagactggccggatcgctgtgaacgggtccgtattttgctaagagcagtagcctttgaacttagcatatgcatcgaaccctcggagcaaagtcgtttggccgcagcattagtacgtttgcgtcgtttgctgttattccttggccttgaaaaagagtgccagcgtgaggagtggatttgccagttgccgcctaatacattactgccgctactactcgatattatttgtgagcgctggcttttcagtgattggttgcttgatagacttaccgctatagtttcttcatcgaagatgttcaatcggttactccaacaacttgatgcgcagtttatgctgatacccgataactgttttaacgacgaagatcaacgtgaacaaattctcgaaacgcttcgtgaagtaaagataaatcaggttttattctgatacctggctttcaatatttaggtaaattggctttctggctcatcatgaggcgtcaggatggattgggatctcattactgaacgtaatattcagctttttattcaattagcaggattagctgaacggcctttagcaaccaatatgttctggcggcaaggacaatatgaaacctatctaaactatcataacggtcgtattcacttatgtcagatactcaagcaaaccttcttagacgaagaactgctttttaaagcgttggctaactggaaacccgcagcgttccagggtattcctcaacgattatttttgttgcgcgatgggcttgcaatgagttgttctccacctctttccagctccgccgagctctggttacgattacatcatcgacaaataaaatttctggagtcgcaatgcgttcatggttaggtgagggagtcagggcgcaacagtggctcagtgtatgcgcgggtcggcaggatatggttctggcgacggtgttattaatcgctattgtgatgatgctgttacctttgccgacctggatggttgatatcctgattactatcaaccttatgttttcagtgatcctgctcttaattgctatttatcttagtgaccctctcgatttatcggtatttccgtctttattacttattactacattatatcgtttgtcactcacaatcagcacatcacggctggtactgttacaacataatgccggtaatattgtggatgctttcggtaagtttgtcgtaggaggaaatctcaccgttgggttggtcgtatttaccatcattactatcgtgcaatttattgtcattacaaaaggtatcgagagggtggcggaagttagcgcacgtttctcgcttgatgggatgccaggcaaacaaatgagtatcgatggcgatttgcgtgccggagttatcgatgcagaccatgcccgtacattaagacagcatgtccagcaggaaagccgctttctcggtgcgatggacggtgcgatgaaatttgttaaaggcgatacgattgccggtattattgttgttctggtgaacattatcggcggtatcattatcgctatcgtacaatatgatatgtcgatgagtgaggctgttcacacttatagcgtactgtcaatcggagatggtttatgtgggcaaattccatcgctgctgatttcccttagcgcgggaattattgtcacccgtgtcccgggtgagaaacgccagaacctggcgacagagttgagttctcaaattgccagacaacctcagtcgctcatattaaccgctgtggttttaatgctcctcgctttaattcctggctttccttttatcactctcgctttcttttcagcgttgttagcattgccaattatcctcattcgccgcaaaaagtctgtggtttccgcaaatggcgtcgaagcaccggaaaaagatagtatggttcccggcgcatgtcctctaatcttacgtcttagcccgacgttacattctgccgacctgattcgtgatattgacgccatgagatggtttttatttgaggataccggcgtccctctccctgaggtgaatattgaggttttgcctgaacccaccgaaaaattgacggtactgctatatcaggaacccgtatttagtttatctattcccgctcaggcggattatttattgataggcgcggacgctagtgtggtgggtgacagccagacgttaccgaacgggatggggcagatctgttggcttacaaaagacatggcccataaggcgcaaggttttggactggacgttttcgcgggcagccaacgtatctctgccttattaaaatgtgtcctgcttcggcatatgggagagtttattggtgttcaggaaacgcgttatctaatgaatgcgatggaaaaaaactactctgagctggtgaaagagcttcagcgccagttacccattaataaaatcgctgaaactttgcaacggcttgtatcagagcgggtttctattagagatttacgtcttattttcggcaccttaattgactgggcgccacgtgaaaaagatgtcctgatgttgacagaatatgtccgtatcgcgcttcgtcgtcatattctgcgtcgtcttaatccggaaggaaaaccgctgccgattttgcggatcggcgaaggtattgaaaacctcgtgcgtgaatccattcgccagacggcaatggggacctatactgcgctgtcgtctcgtcataagacgcagatcctgcaacttatcgagcaggcgctgaagcagtcagccaaattattcattgtcacttctgtcgacacccgacgtttcttgcgaaaaattacagaagccaccttgttcgacgtaccgattttgtcatggcaggaattaggagaggagagccttatacaagtggtagaaagtattgaccttagcgaagaggagttggcggacaatgaagaatgaattgatgcaacgtctgaggctgaaatatccgccccccgatggttattgtcgatggggccgaattcaggatgtcagcgcaacgttgttaaatgcgtggttgcctggggtatttatgggcgagttgtgctgtataaagcctggagaagaacttgctgaagtcgtggggattaatggcagcaaagctttgctatctccttttacgagtacaatcgggcttcactgcgggcagcaagtgatggccttaaggcgacgccatcaggttcccgtgggcgaagcgttattagggcgagttattgatggctttggtcgtccccttgatggccgcgaactgcccgacgtctgctggaaagactatgatgcaatgcctcctcccgcaatggttcgacagcctatcactcaaccattaatgacggggattcgcgctattgatagcgttgcgacctgtggcgaagggcaacgagtgggtattttttctgctcctggcgtggggaaaagcacgcttctggcgatgctgtgtaatgcgccagacgcagacagcaatgttctggtgttaattggtgaacgtggacgagaagtccgcgaattcatcgattttacactgtctgaagagacccgaaaacgttgtgtcattgttgtcgcaacctctgacagacccgccttagagcgcgtgagggcgctgtttgtggccaccacgatagcagaattttttcgcgataatggaaagcgagtcgtcttgcttgccgactcactgacgcgttatgccagggccgcacgggaaatcgctctggccgccggagagaccgcggtttctggagaatatccgccaggcgtatttagtgcattgccacgacttttagaacgtacgggaatgggagaaaaaggcagtattaccgcattttatacggtactggtggaaggcgatgatatgaatgagccgttggcggatgaagtccgttcactgcttgatggacatattgtactatcccgacggcttgcagagagggggcattatcctgccattgacgtgttggcaacgctcagccgcgtttttccagtcgttaccagccatgagcatcgtcaactggcggcgatattgcgacggtgcctggcgctttaccaggaggttgaactgttaatacgcattggggaataccagcgaggagttgatacagatactgacaaagccattgatacctatccggatatttgcacatttttgcgacaaagtaaggatgaagtatgcggacccgagctacttatagaaaaattacaccaaatactcaccgagtgatcatggaaactttgctggagataatcgcgcggcgtgaaaagcaattacgcggcaagcttaccgtacttgatcagcagcaacaggcgattattacggaacagcagatttgccagacgcgcgctttagcagtgtctaccagactgaaagaattaatgggctggcaaggtacgttatcttgtcatttattgttggataagaaacaacaaatggccgggttattcactcaggcgcagagctttttgacgcaacggcagcagttagagaatcagtatcagcagcttgtctcccggcgaagcgaattacagaagaattttaatgcgcttatgaaaaagaaagaaaaaattactatggtattaagcgatgcgtattaccaaagttgagggaagtcttgggttgccatgccagtcttatcaggatgataacgaggcggaggcggaacgtatggactttgaacaactcatgcaccaggcattacccattggtgagaataatcctcctgcagcattgaataagaacgtggttttcacgcaacgttatcgtgttagtggcggttatcttgacggtgtagagtgtgaagtatgtgaatcaggggggctaatccagttaagaatcaatgtccctcatcatgaaatttaccgttcgatgaaagcgctaaagcagtggctggagtctcagttgctgcatatggggtatataatttccctggagatattctatgttaagaatagcgaatgaagagcgtccgtgggtggagatacttccaacgcaaggcgctaccattggtgagctgacattgagtatgcaacaatatccagtacagcaagggacattatttaccataaattatcataatgagctgggtagggtgtggattgcagaacaatgctggcagcgctggtgtgaagggctaattggcaccgctaatcgatcggctatcgatcctgaattgctatatggaatagctgaatgggggctggcgccgttattgcaagccagtgatgcaaccctctgtcagaacgagccgccaacatcctgcagtaatctaccacatcagctagcgttgcatattaaatggacagttgaagagcatgagttccatagcattatttttacatggccaacgggttttttgcgcaatatagtcggagagctttctgctgagcgacaacagatttatcctgcccctcctgtggtagtccctgtatattcaggctggtgccagcttacattaatcgaacttgagtctatcgaaatcggcatgggcgttcggattcattgcttcggcgacatcagactcggtttttttgctattcaactacctgggggaatctacgcaagggtgttgctgacagaggataacacgatgaaatttgacgaattagtccaggatatcgaaacgctacttgcgtcagggagcccaatgtcaaagagtgacggaacgtcttcagtcgaacttgagcagataccacaacaggtgctctttgaggtcggacgtgcgagtctggaaattggacaattacgacaacttaaaacgggggacgttttgcctgtaggtggatgttttgcgccagaggtgacgataagagtaaatgaccgtattattgggcaaggtgagttgattgcctgtggcaatgaatttatggtgcgtattacacgttggtatctttgcaaaaatacagcgtaaacctgataagaaaaataatatgcgaacaatataatagcgttccaggtcgtgtcatgagagatacagtatgtctttacccgattcgcctttgcaactgattggtatattgtttctgctttcaatactgcctctcattatcgtcatgggaacttctttccttaaactggcggtggtattttcgattttacgaaatgctctgggtattcaacaagtccccccaaatatcgcactgtatggccttgcgcttgtactttccttattcattatggggccgacgctattagctgtaaaagagcgctggcatccggttcaggtcgctggcgctcctttctggacgtctgagtgggacagtaaagcattagcgccttatcgacagtttttgcaaaaaaactctgaagagaaggaagccaattattttcggaatttgataaaacgaacctggcctgaagacataaaaagaaagataaaacctgattctttgctcatattaattccggcatttacggtgagtcagttaacgcaggcatttcggattggattacttatttatcttccctttctggctattgacctgcttatttcaaatatactgctggctatggggatgatgatggtgtcgccgatgaccatttcattaccgtttaagctgctaatatttttactggcaggcggttgggatctgacactggcgcaattggtacagagcttttcatgaatgattctgaattgacgcaatttgtaacgcaacttttatggatcgtcctttttacgtctatgccggtagtgttggtggcatcggtagttggtgtcatcgtaagccttgttcaggccttgactcaaatacaggaccaaacgctacagttcatgattaaattattggcaattgcaataaccttaatggtcagctacccatggcttagcggtatcctgttgaattatacccggcagataatgttacgaattggagagcatggttgaatggcacaacaggtaaatgagtggcttattgcattggctgtggcttttattcgaccattgagcctttctttattacttcccttattaaaaagtggcagtttaggggccgcacttttacgtaatggcgtgcttatgtcacttacctttccgatattaccaatcatttaccagcagaagattatgatgcatattggtaaagattacagttggttagggttagtcactggagaggtgattattggtttttcaattgggttttgtgcggcggttcccttttgggccgttgatatggcggggtttctgcttgatactttacgtggcgcgacaatgggtacgatattcaattctacaatagaagctgaaacctcactttttggcttgcttttcagccagttcttgtgtgttattttctttataagcggcggcatggagtttatattaaacattctgtatgagtcatatcaatatttaccaccagggcgtactttattatttgaccagcaatttttaaaatatatccaggcagagtggagaacgctttatcaattatgtatcagcttctctcttcctgccataatatgtatggtattagccgatctggctttaggtcttttaaatcggtcggcacaacaattgaatgtgtttttcttctcaatgccgctcaaaagtatattggttctactgacgctcctgatctcattcccttatgctcttcatcactatttggttgaaagcgataaattttatatttatctaaaagactggtttccatctgtatgagcgagaaaacagaacagcctacagaaaagaaattacgtgatggccgtaaggaagggcaggttgtcaaaagtattgaaataacatcattatttcagctgattgcgctttatttgtattttcatttctttactgaaaagatgattttgatactgattgagtcaataactttcacattacaattagtaaataaaccattttcttatgcattaacgcaattgagtcatgctttaatagagtcactgacttctgcactgctgtttctgggcgctggggtaatagttgctactgtgggtagcgtgtttcttcaggtgggggtggttattgccagcaaggccattggttttaaaagcgagcatataaatccggtaagtaattttaagcagatattctctttacatagcgtagtagaattatgtaaatccagcctaaaagttatcatgctatctcttatctttgcctttttcttttattattatgccagtacttttcgggcgctaccgtactgtgggttagcctgtggcgtgcttgtggtttcttctttaataaaatggttatgggtaggggtgatggttttttatatcgtcgttggcatactggactattcttttcaatattataagattagaaaagatctaaaaatgagtaaagatgacgtaaaacaggagcataaagatctggagggcgaccctcaaatgaagacgcggcgtcgggaaatgcagagtgaaatacaaagtgggagtttagctcaatctgttaaacaatctgttgcggtagtgcgtaatccaacgcatattgcggtttgtcttggctatcatcccaccgatatgccaataccacgcgtcctggaaaaaggcagtgatgctcaagctaactatattgttaacatcgctgaacgcaactgcatccccgttgttgaaaatgttgagctggcccgctcattattttttgaagtggaacgcggagataaaattcctgaaacgttatttgaacccgttgcagccttgttacgtatggtgatgaagatagattatgcgcattctaccgaaacaccataaatgcttttggtatgcttcttcaggccactgcgaagg

SEQ ID NO: 3 - DNA, 59 bp, Artificial Sequence
  hilD forward primer
tttgtaagtaatagtcatcagcgtcctgccgcagataacttgtaggctggagctgcttc

SEQ ID NO: 4 - DNA, 59 bp, Artificial Sequence
  hilD reverse primer
agcttccactgtctactgggtgacgaagatataatgttgtcatatgaatatcctcctta

SEQ ID NO: 5 - DNA, 59 bp, Artificial Sequence
  SPI-1 forward primer
taattatatcatgatgagttcagccaacggtgatatggcctgtaggctggagctgcttc

SEQ ID NO: 6 - DNA, 59 bp, Artificial Sequence
  SPI-1 reverse primer
gctggaaggatttcctctggcaggcaaccttataatttcacatatgaatatcctcctta

SEQ ID NO: 7 - DNA, 59 bp, Artificial Sequence
  SPI-2 forward primer
tgcttaataccatcggacgcccctggttaatactctattatgtaggctggagctgcttc

SEQ ID NO: 8 - DNA, 59 bp, Artificial Sequence
  SPI-2 reverse primer
ctgaagaagcataccaaaagcatttatggtgtttcggtagcatatgaatatcctcctta

SEQ ID NO: 9 - DNA, 46 bp, Artificial Sequence
  EcoRI(pJL39 plasmid) forward primer
cggaattcaccatgtctagattagataaaagtaaagtgattaacag

SEQ ID NO: 10 - DNA, 48 bp, Artificial Sequence
  PvuII-XbaI(pJL39 plasmid) reverse primer
gctctagacagctgttaagacccactttcacatttaagttgtttttct

SEQ ID NO: 11 - DNA, 39 bp, Artificial Sequence
  pSF-OXB1 forward primer
ctactccgtcaagccgtcaagctgttgtgaccgcttgct

SEQ ID NO: 12 - DNA, 57 bp, Artificial Sequence
  pSF-OXB1 reverse primer
tgaattcctcctgctagctagttggtaacgaatcagacgccgggtaataccggatag

SEQ ID NO: 13 - DNA, 28 bp, Artificial Sequence
  Cytolysin A forward primer
agtccatggttatgaccggaatatttgc

SEQ ID NO: 14 - DNA, 29 bp, Artificial Sequence
  Cytolysin A reverse primer
gatgtttaaactcagacgtcaggaacctc

SEQ ID NO: 15 - DNA, 912 bp, Unknown
  Cytolysin A gene
atgaccggaatatttgcagaacaaactgtagaggtagttaaaagcgcgatcgaaaccgcagacggggcattagatctttataacaaatacctcgaccaggtcatcccctggaagacctttgatgaaaccataaaagagttaagccgttttaaacaggagtactcgcaggaagcttctgttttagttggtgatattaaagttttgcttatggacagccaggacaagtattttgaagcgacacaaactgtttatgaatggtgtggtgtcgtgacgcaattactctcagcgtatattttactatttgatgaatataatgagaaaaaagcatcagcccagaaagacattctcattaggatattagatgatggtgtcaagaaactgaatgaagcgcaaaaatctctcctgacaagttcacaaagtttcaacaacgcttccggaaaactgctggcattagatagccagttaactaatgatttttcggaaaaaagtagttatttccagtcacaggtggatagaattcgtaaggaagcttatgccggtgctgcagccggcatagtcgccggtccgtttggattaattatttcctattctattgctgcgggcgtgattgaagggaaattgattccagaactgaataacaggctaaaaacagtgcaaaatttctttactagcttatcagctacagtgaaacaagcgaataaagatatcgatgcggcaaaattgaaattagccactgaaatagcagcaattggggagataaaaacggaaaccgaaacaaccagattctacgttgattatgatgatttaatgctttctttattaaaaggagctgcaaagaaaatgattaacacctgtaatgaataccaacaaagacacggtaagaagacgcttttcgaggttcctgacgtctaa